European Patent Application EP 4 332 235 A1, published March 6, 2024. Title: HIGHLY SENSITIVE METHODS FOR ACCURATE PARALLEL QUANTIFICATION OF VARIANT NUCLEIC ACIDS. Applicant: Genomill Health Oy. The sequence listing filed with the application follows.

SEQUENCE LISTING (28 sequences)

SEQ ID NO: 1 - DNA, 31 bp, synthetic construct
  source 1..31: mol_type = other DNA
ggggcccgccgtcgatcggagccgttaggat

SEQ ID NO: 2 - DNA, 31 bp, synthetic construct
  source 1..31: mol_type = other DNA
ttaaggtgccgtcgatcggagccgacgtacg

SEQ ID NO: 3 - DNA, 31 bp, synthetic construct; identical to SEQ ID NO: 2
  source 1..31: mol_type = other DNA

SEQ ID NO: 4 - DNA, 31 bp, synthetic construct
  source 1..31: mol_type = other DNA
tataatagaggtcgtgcagtcacgacccggt

SEQ ID NO: 5 - DNA, 31 bp, synthetic construct
  source 1..31: mol_type = other DNA
accaggtgccgtcgatcggagccgacccggt

SEQ ID NO: 6 - DNA, 31 bp, synthetic construct
  source 1..31: mol_type = other DNA
gggccgggaggtcgtgcagtcacgttaggat

SEQ ID NO: 7 - DNA, 31 bp, synthetic construct
  source 1..31: mol_type = other DNA
tccaggtgagtcgatccgtcacgtacgtacg

SEQ ID NO: 8 - DNA, 31 bp, synthetic construct
  source 1..31: mol_type = other DNA
aaaattttagcgtacgtcgtacgtttaggat

SEQ ID NO: 9 - DNA, 31 bp, synthetic construct; identical to SEQ ID NO: 4
  source 1..31: mol_type = other DNA

SEQ ID NO: 10 - DNA, 31 bp, synthetic construct
  source 1..31: mol_type = other DNA
aggaccttgagtcgatccgcacgtacccggt

SEQ ID NO: 11 - DNA, 31 bp, synthetic construct
  source 1..31: mol_type = other DNA
agcgaccgaggtcgtgcagtcacgacgtacg

SEQ ID NO: 12 - DNA, 31 bp, synthetic construct; identical to SEQ ID NO: 4
  source 1..31: mol_type = other DNA

SEQ ID NO: 13 - DNA, 31 bp, synthetic construct
  source 1..31: mol_type = other DNA
ggaaaaagccgtcgatcggagccgttaggat

SEQ ID NO: 14 - DNA, 31 bp, synthetic construct
  source 1..31: mol_type = other DNA
atatacagaggtcgtgcagtcacgttaggat

SEQ ID NO: 15 - DNA, 31 bp, synthetic construct
  source 1..31: mol_type = other DNA
gagagccgaggtcgtgcagtcacgacccggt

SEQ ID NO: 16 - DNA, 31 bp, synthetic construct
  source 1..31: mol_type = other DNA
cgcacgcgaggtcgtgcagtcacgacgtacg

SEQ ID NO: 17 - DNA, 31 bp, synthetic construct
  source 1..31: mol_type = other DNA
attacaagccgtcgatcggagccgacccggt

SEQ ID NO: 18 - DNA, 31 bp, synthetic construct; identical to SEQ ID NO: 4
  source 1..31: mol_type = other DNA

SEQ ID NO: 19 - DNA, 31 bp, synthetic construct
  source 1..31: mol_type = other DNA
gggcaattagcgtacgtcgtacgtacgtacg

SEQ ID NO: 20 - DNA, 31 bp, synthetic construct
  source 1..31: mol_type = other DNA
tatgcgagccgtcgatcggagccgacgtacg

SEQ ID NO: 21 - DNA, 31 bp, synthetic construct; identical to SEQ ID NO: 10
  source 1..31: mol_type = other DNA

SEQ ID NO: 22 - DNA, 31 bp, synthetic construct; identical to SEQ ID NO: 17
  source 1..31: mol_type = other DNA

SEQ ID NO: 23 - DNA, 31 bp, synthetic construct
  source 1..31: mol_type = other DNA
gaagaattagcgtacgtcgtacgtttaggat

SEQ ID NO: 24 - DNA, 31 bp, synthetic construct; identical to SEQ ID NO: 23
  source 1..31: mol_type = other DNA

SEQ ID NO: 25 - DNA, 31 bp, synthetic construct; identical to SEQ ID NO: 19
  source 1..31: mol_type = other DNA

SEQ ID NO: 26 - DNA, 31 bp, synthetic construct
  source 1..31: mol_type = other DNA
gagcacttagcgtacgtcgtacgtacccggt

SEQ ID NO: 27 - DNA, 31 bp, synthetic construct
  source 1..31: mol_type = other DNA
aaaggggcgagtcgatccgcacgtttaggat

SEQ ID NO: 28 - DNA, 31 bp, synthetic construct
  source 1..31: mol_type = other DNA
agcgcgcgccgtcgatcggagccgttaggat